European Patent Application EP 4 265 630 A1, published October 25, 2023. Title: ANTI-INFLAMMATORY PEPTIDE FOR PREVENTING OR TREATING ATOPIC DERMATITIS. Applicant: AJOU UNIVERSITY INDUSTRY-ACADEMIC COOPERATION FOUNDATION. The sequence listing filed with the application follows.

SEQUENCE LISTING (16 sequences)

SEQ ID NO: 1 - protein, 12 aa, Artificial Sequence
  peptide-A900
GCVTVLRCGEIV

SEQ ID NO: 2 - protein, 12 aa, Artificial Sequence
  peptide-A901
GCETVLRCGEIV

SEQ ID NO: 3 - protein, 12 aa, Artificial Sequence
  peptide-A902
GCVTELRCGEIV

SEQ ID NO: 4 - protein, 12 aa, Artificial Sequence
  peptide-A903
GCETELRCGEIV

SEQ ID NO: 5 - protein, 12 aa, Artificial Sequence
  peptide-A904
GCVSVLRCGEIV

SEQ ID NO: 6 - protein, 12 aa, Artificial Sequence
  peptide-A905
GCVSVLRCGEIV

SEQ ID NO: 7 - protein, 12 aa, Artificial Sequence
  peptide-A906
GCVTVLLCGEIV

SEQ ID NO: 8 - protein, 12 aa, Artificial Sequence
  peptide-A907
GCESEILCGEIV

SEQ ID NO: 9 - protein, 8 aa, Artificial Sequence
  peptide-A909
GCVCGEIV

SEQ ID NO: 10 - protein, 9 aa, Artificial Sequence
  peptide-A910
GCVTCGEIV

SEQ ID NO: 11 - protein, 10 aa, Artificial Sequence
  peptide-A911
GCVTVCGEIV

SEQ ID NO: 12 - protein, 11 aa, Artificial Sequence
  peptide-A912
GCVTVLCGEIV

SEQ ID NO: 13 - protein, 8 aa, Artificial Sequence
  peptide-A913
GCRCGEIV

SEQ ID NO: 14 - protein, 9 aa, Artificial Sequence
  peptide-A914
GCLRCGEIV

SEQ ID NO: 15 - protein, 10 aa, Artificial Sequence
  peptide-A915
GCVLRCGEIV

SEQ ID NO: 16 - protein, 11 aa, Artificial Sequence
  peptide-A916
GCTVLRCGEIV